European Patent Specification EP 3 949 995 B1, published June 19, 2024. Title: PEPTIDE AND USE THEREOF. Applicant: NIIGATA UNIVERSITY. The sequence listing filed with the application follows.

SEQUENCE LISTING (14 sequences)

SEQ ID NO: 1 - protein, 9 aa, Artificial Sequence
  Synthesized
KCAELFRHL

SEQ ID NO: 2 - protein, 9 aa, Artificial Sequence
  Synthesized
WPPLQRWRN

SEQ ID NO: 3 - protein, 9 aa, Artificial Sequence
  Synthesized
RTHPVWSRT

SEQ ID NO: 4 - protein, 9 aa, Artificial Sequence
  Synthesized
RRWMQWPWH

SEQ ID NO: 5 - protein, 19 aa, Artificial Sequence
  Synthesized
KCAELFRHLGKCAELFRHL

SEQ ID NO: 6 - protein, 19 aa, Artificial Sequence
  Synthesized
  MISC_FEATURE (2)..(2): Xaa indicates Methyl-Cys.
  MISC_FEATURE (12)..(12): Xaa indicates Methyl-Cys.
KXAELFRHLGKXAELFRHL

SEQ ID NO: 7 - DNA, 27 bp, Artificial Sequence
  Synthesized
aagtgcgccgagctgttccggcacctg

SEQ ID NO: 8 - DNA, 27 bp, Artificial Sequence
  Synthesized
tggccccccctgcagcggtggcggaac

SEQ ID NO: 9 - DNA, 27 bp, Artificial Sequence
  Synthesized
cggacccaccccgtgtggtcccggacc

SEQ ID NO: 10 - DNA, 27 bp, Artificial Sequence
  Synthesized
cggcggtggatgcagtggccctggcac

SEQ ID NO: 11 - DNA, 57 bp, Artificial Sequence
  Synthesized
aagtgcgccgagctgttccggcacctgggcaagtgcgccgagctgttccggcacctg

SEQ ID NO: 12 - protein, 9 aa, Artificial Sequence
  Synthesized
RRRRRRRRR

SEQ ID NO: 13 - protein, 9 aa, Artificial Sequence
  Synthesized
RARVAWDWI

SEQ ID NO: 14 - protein, 9 aa, Artificial Sequence
  Synthesized
WTRTQWPLH